European Patent Specification EP 3 694 535 B1, published November 26, 2025. Title: PORCINE G-CSF VARIANTS AND THEIR USES. Applicant: Elanco US Inc. Ambrx Inc. The sequence listing filed with the application follows.

SEQUENCE LISTING (13 sequences)

SEQ ID NO: 1 - protein, 175 aa, Sus scrofa
MAPLSPASSLPQSFLLKCLEQVRKIQADGAELQERLCATHKLCHPQELVLLGHSLGLPQASLSSCSSQALQLTGCLNQLHGGLVLYQGLLQALAGISPELAPALDILQLDVTDLATNIWLQMEDLRMAPASLPTQGTVPTFTSAFQRRAGGVLVVSQLQSFLELAYRVLRYLAEP

SEQ ID NO: 2 - protein, 175 aa, Artificial Sequence
  Synthetic
  MISC_FEATURE (44)..(44): Xaa is para-acetylphenylalanine
MAPLSPASSLPQSFLLKCLEQVRKIQADGAELQERLCATHKLCXPQELVLLGHSLGLPQASLSSCSSQALQLTGCLNQLHGGLVLYQGLLQALAGISPELAPALDILQLDVTDLATNIWLQMEDLRMAPASLPTQGTVPTFTSAFQRRAGGVLVVSQLQSFLELAYRVLRYLAEP

SEQ ID NO: 3 - protein, 174 aa, Sus scrofa
APLSPASSLPQSFLLKCLEQVRKIQADGAELQERLCATHKLCHPQELVLLGHSLGLPQASLSSCSSQALQLTGCLNQLHGGLVLYQGLLQALAGISPELAPALDILQLDVTDLATNIWLQMEDLRMAPASLPTQGTVPTFTSAFQRRAGGVLVVSQLQSFLELAYRVLRYLAEP

SEQ ID NO: 4 - protein, 174 aa, Artificial Sequence
  Synthetic
  MISC_FEATURE (43)..(43): Xaa is para-acetylphenylalanine
APLSPASSLPQSFLLKCLEQVRKIQADGAELQERLCATHKLCXPQELVLLGHSLGLPQASLSSCSSQALQLTGCLNQLHGGLVLYQGLLQALAGISPELAPALDILQLDVTDLATNIWLQMEDLRMAPASLPTQGTVPTFTSAFQRRAGGVLVVSQLQSFLELAYRVLRYLAEP

SEQ ID NO: 5 - DNA, 528 bp, Sus scrofa
atggcccctctcagccctgccagctccctgccccagagcttcctgctcaagtgcttagagcaagtgaggaaaatccaggctgatggcgccgagctgcaggagaggctgtgtgccacccacaagctgtgccacccccaggagctggtgctgctcgggcactctctgggcctcccccaggcttccctgagcagctgctccagccaggccctgcagctgactggctgcctgaaccaactgcatggcggcctcgtcctctaccagggcctcctgcaggccctggcgggcatctccccagagctggcccccgccctggacatactgcagctggatgtcaccgacttagccaccaacatctggctgcagatggaagacctgaggatggccccggcctcgcttcccacccagggcaccgtgccgaccttcacctcggccttccagcgccgggcaggaggggtcctggttgtctcccagctgcagagcttcctggagctggcgtaccgtgtcctgcgctacctcgccgagccctga

SEQ ID NO: 6 - DNA, 528 bp, Artificial Sequence
  synthetic cDNA encodes SEQ ID NOs: 2 & 4
atggcccctctcagccctgccagctccctgccccagagcttcctgctcaagtgcttagagcaagtgaggaaaatccaggctgatggcgccgagctgcaggagaggctgtgtgccacccacaagctgtgctagccccaggagctggtgctgctcgggcactctctgggcctcccccaggcttccctgagcagctgctccagccaggccctgcagctgactggctgcctgaaccaactgcatggcggcctcgtcctctaccagggcctcctgcaggccctggcgggcatctccccagagctggcccccgccctggacatactgcagctggatgtcaccgacttagccaccaacatctggctgcagatggaagacctgaggatggccccggcctcgcttcccacccagggcaccgtgccgaccttcacctcggccttccagcgccgggcaggaggggtcctggttgtctcccagctgcagagcttcctggagctggcgtaccgtgtcctgcgctacctcgccgagccctga

SEQ ID NO: 7 - protein, 175 aa, Artificial Sequence
  Synthetic
  MISC_FEATURE (1)..(1): Xaa is norleucine or methionine
  MISC_FEATURE (44)..(44): Xaa is para-acetylphenylalanine
  MISC_FEATURE (122)..(122): Xaa is norleucine or methionine
  MISC_FEATURE (127)..(127): Xaa is norleucine or methionine
XAPLSPASSLPQSFLLKCLEQVRKIQADGAELQERLCATHKLCXPQELVLLGHSLGLPQASLSSCSSQALQLTGCLNQLHGGLVLYQGLLQALAGISPELAPALDILQLDVTDLATNIWLQXEDLRXAPASLPTQGTVPTFTSAFQRRAGGVLVVSQLQSFLELAYRVLRYLAEP

SEQ ID NO: 8 - protein, 173 aa, Artificial Sequence
  Synthetic
  MISC_FEATURE (42)..(42): Xaa is para-acetylphenylalanine
PLSPASSLPQSFLLKCLEQVRKIQADGAELQERLCATHKLCXPQELVLLGHSLGLPQASLSSCSSQALQLTGCLNQLHGGLVLYQGLLQALAGISPELAPALDILQLDVTDLATNIWLQMEDLRMAPASLPTQGTVPTFTSAFQRRAGGVLVVSQLQSFLELAYRVLRYLAEP

SEQ ID NO: 9 - protein, 175 aa, Artificial Sequence
  Synthetic
  MISC_FEATURE (44)..(44): Xaa is para-acetylphenylalanine
MAPLSPASSLPQSFLLKSLEQVRKIQADGAELQERLCATHKLCXPQELVLLGHSLGLPQASLSSCSSQALQLTGCLNQLHGGLVLYQGLLQALAGISPELAPALDILQLDVTDLATNIWLQMEDLRMAPASLPTQGTVPTFTSAFQRRAGGVLVVSQLQSFLELAYRVLRYLAEP

SEQ ID NO: 10 - protein, 175 aa, Artificial Sequence
  Synthetic
  MISC_FEATURE (1)..(1): Xaa is norleucine or methionine
  MISC_FEATURE (44)..(44): Xaa is para-acetylphenylalanine
  MISC_FEATURE (122)..(122): Xaa is norleucine or methionine
  MISC_FEATURE (127)..(127): Xaa is norleucine or methionine
XAPLSPASSLPQSFLLKSLEQVRKIQADGAELQERLCATHKLCXPQELVLLGHSLGLPQASLSSCSSQALQLTGCLNQLHGGLVLYQGLLQALAGISPELAPALDILQLDVTDLATNIWLQXEDLRXAPASLPTQGTVPTFTSAFQRRAGGVLVVSQLQSFLELAYRVLRYLAEP

SEQ ID NO: 11 - protein, 174 aa, Artificial Sequence; identical to SEQ ID NO: 4
  Synthetic
  MISC_FEATURE (43)..(43): Xaa is para-acetylphenylalanine

SEQ ID NO: 12 - protein, 173 aa, Artificial Sequence
  Synthetic
  MISC_FEATURE (42)..(42): Xaa is para-acetylphenylalanine
PLSPASSLPQSFLLKSLEQVRKIQADGAELQERLCATHKLCXPQELVLLGHSLGLPQASLSSCSSQALQLTGCLNQLHGGLVLYQGLLQALAGISPELAPALDILQLDVTDLATNIWLQMEDLRMAPASLPTQGTVPTFTSAFQRRAGGVLVVSQLQSFLELAYRVLRYLAEP

SEQ ID NO: 13 - protein, 174 aa, Artificial Sequence
  Synthetic
  misc_feature (1)..(1): Xaa can be any naturally occurring amino acid
  misc_feature (17)..(17): Xaa can be any naturally occurring amino acid
  MISC_FEATURE (43)..(43): Xaa is para-acetylphenylalanine
  misc_feature (121)..(121): Xaa can be any naturally occurring amino acid
  misc_feature (126)..(126): Xaa can be any naturally occurring amino acid
XPLSPASSLPQSFLLKXLEQVRKIQADGAELQERLCATHKLCXPQELVLLGHSLGLPQASLSSCSSQALQLTGCLNQLHGGLVLYQGLLQALAGISPELAPALDILQLDVTDLATNIWLQXEDLRXAPASLPTQGTVPTFTSAFQRRAGGVLVVSQLQSFLELAYRVLRYLAEP